European Patent Specification EP 3 321 380 B1, published September 6, 2023. Title: METHODS FOR THE DIAGNOSIS OF BACTERIAL VAGINOSIS. Applicant: QUEST DIAGNOSTICS INVESTMENTS INCORPORATED. Application PCT/US2010/056983. The sequence listing filed with the application follows.

SEQUENCE LISTING (22 sequences)

SEQ ID NO: 1 - DNA, 20 bp, Artificial Sequence
  Description of Artificial Sequence: Synthetic primer
tgccccatagtctgggatac

SEQ ID NO: 2 - DNA, 20 bp, Artificial Sequence
  Description of Artificial Sequence: Synthetic primer
atgtggccgatcagtctctc

SEQ ID NO: 3 - DNA, 25 bp, Artificial Sequence
  Description of Artificial Sequence: Synthetic probe
ccggataagaaagcagatcgcatga

SEQ ID NO: 4 - DNA, 20 bp, Artificial Sequence
  Description of Artificial Sequence: Synthetic primer
agtaacgcgtgggtaacctg

SEQ ID NO: 5 - DNA, 20 bp, Artificial Sequence
  Description of Artificial Sequence: Synthetic primer
gtccatcctttagcgacagc

SEQ ID NO: 6 - DNA, 25 bp, Artificial Sequence
  Description of Artificial Sequence: Synthetic probe
ccggataaaagctactttcgcatga

SEQ ID NO: 7 - DNA, 25 bp, Artificial Sequence
  Description of Artificial Sequence: Synthetic probe
ccggataagaaagcagatcgcatga

SEQ ID NO: 8 - DNA, 19 bp, Artificial Sequence
  Description of Artificial Sequence: Synthetic primer
acacggcccaaactcctac

SEQ ID NO: 9 - DNA, 20 bp, Artificial Sequence
  Description of Artificial Sequence: Synthetic primer
cgatccgaaaaccttcttca

SEQ ID NO: 10 - DNA, 24 bp, Artificial Sequence
  Description of Artificial Sequence: Synthetic probe
ccgaatgatgcaatcaacttcgag

SEQ ID NO: 11 - DNA, 20 bp, Artificial Sequence
  Description of Artificial Sequence: Synthetic primer
taggggagcgaacaggatta

SEQ ID NO: 12 - DNA, 20 bp, Artificial Sequence
  Description of Artificial Sequence: Synthetic primer
cccgtcaattcctttgagtt

SEQ ID NO: 13 - DNA, 25 bp, Artificial Sequence
  Description of Artificial Sequence: Synthetic probe
tggggagattatactttccgtgccg

SEQ ID NO: 14 - DNA, 20 bp, Artificial Sequence
  Description of Artificial Sequence: Synthetic primer
cacattgggactgagacacg

SEQ ID NO: 15 - DNA, 20 bp, Artificial Sequence
  Description of Artificial Sequence: Synthetic primer
acgcttgccacctacgtatt

SEQ ID NO: 16 - DNA, 25 bp, Artificial Sequence
  Description of Artificial Sequence: Synthetic probe
acggtaccgtaagagaaagccacgg

SEQ ID NO: 17 - DNA, 20 bp, Artificial Sequence
  Description of Artificial Sequence: Synthetic primer
ctcttggaaacgggtggtaa

SEQ ID NO: 18 - DNA, 20 bp, Artificial Sequence
  Description of Artificial Sequence: Synthetic primer
gagtctgggccgtatctcag

SEQ ID NO: 19 - DNA, 23 bp, Artificial Sequence
  Description of Artificial Sequence: Synthetic probe
agcttgtaggcggggtaatggcc

SEQ ID NO: 20 - DNA, 20 bp, Artificial Sequence
  Description of Artificial Sequence: Synthetic primer
gagtaacacgtgggcaacct

SEQ ID NO: 21 - DNA, 20 bp, Artificial Sequence
  Description of Artificial Sequence: Synthetic primer
gcccatcctgaagtgatagc

SEQ ID NO: 22 - DNA, 25 bp, Artificial Sequence
  Description of Artificial Sequence: Synthetic probe
ctgaagcgggggataacatctggaa